European Patent Application EP 4 257 978 A1, published October 11, 2023. Title: Method for screening a candidate molecule which can form a complex with multiple target molecules. Applicant: CHUGAI SEIYAKU KABUSHIKI KAISHA. The sequence listing filed with the application follows.

SEQUENCE LISTING (124 sequences)

SEQ ID NO: 1 - protein, 15 aa, Artificial Sequence
  Avi-tag sequence
GLNDIFEAQKIEWHE

SEQ ID NO: 2 - protein, 7 aa, Artificial Sequence
  TEV protease sequence
ENLYFQG

SEQ ID NO: 3 - protein, 6 aa, Artificial Sequence
  His tag sequence
HHHHHH

SEQ ID NO: 4 - DNA, 38 bp, Artificial Sequence
  Fw(GFP)
gtaatacgactcactatagggttaactttaagaaggag

SEQ ID NO: 5 - DNA, 28 bp, Artificial Sequence
  Rv(GFP)
tttttttagagccagagccagagccaga

SEQ ID NO: 6 - DNA, 41 bp, Artificial Sequence
  reverse transcription S2_mRNA#13
tttgtccccgccgccctatcgccggtgccggtgccggtcgg

SEQ ID NO: 7 - DNA, 33 bp, Artificial Sequence
  Fw_1for SNAP(N) prep.
taaggagatataaatatggacaaagactgcgaa

SEQ ID NO: 8 - DNA, 50 bp, Artificial Sequence
  Rv_1for SNAP(N) prep.
agagccagagccagagccagagccagagccctgctggaacactgggtggt

SEQ ID NO: 9 - DNA, 52 bp, Artificial Sequence
  Fw_2 for SNAP(N) prep.
ggcgtaatacgactcactatagggttaactttaataaggagatataaatatg

SEQ ID NO: 10 - DNA, 37 bp, Artificial Sequence
  Rv_2 for SNAP(N) prep.
tttttttagagccagagccagagccagagccagagcc

SEQ ID NO: 11 - DNA, 44 bp, Artificial Sequence
  Fw_1for SNAP(C) prep.
taaggagatataaatatggtcgacgagagctttacccgccaggt

SEQ ID NO: 12 - DNA, 51 bp, Artificial Sequence
  Rv_1for SNAP(C) prep.
agagccagagccagagccagagccagagccattaacctcgagtttaaacgc

SEQ ID NO: 13 - DNA, 33 bp, Artificial Sequence
  GGSS-primer_F
tggtggcagcagcagcaagggcgaggaactgtt

SEQ ID NO: 14 - DNA, 34 bp, Artificial Sequence
  GGSS-primer_R
ctgctgctgccaccatgatggtgatgatggtgac

SEQ ID NO: 15 - DNA, 852 bp, Artificial Sequence
  GFP1-9
catatgggtggcaccagcagcaagggcgaggaactgttcaccggtgtggttccgatcctggtggagctggacggcgatgttaacggtcacaaatttagcgtgcgtggtgagggcgaaggtgacgcgaccatcggcaagctgaccctgaaattcattagcaccaccggtaaactgccggtgccgtggccgaccctggttaccaccctgacctacggtgtgcaggcgtttagccgttatccggaccacatgaagcgtcacgatttctttaaaagcgcgatgccggagggctacgttcaagaacgtaccattagcttcaaggacgatggcaagtataaaacccgtgcggtggttaaatttgagggcgataccctggttaaccgtatcgagctgaagggtaccgacttcaaagaagatggcaacattctgggtcacaagctggaatacaactttaacagccacaacgtgtatatcaccgcggacaagcagaaaaacggcattaaagcgaacttcaccgtgcgtcacaacgttgaggacggtagcgttcaactggcggatcactaccagcaaaacaccccgattggtgatggtacccgtggcagcggtagcattgaaggtcgtcatagcggcagcggtagcccggtgctgctgccggacaaccactatctgagcacccagaccgttctgagcaaagatccgaacgaggcgggcactcgtggcagcggtagcatcgaaggtcgtcacagcggcagcggtagccgtgaccacatggtgctgcacgaatacgttaacgcggcgggcatcacccacggtatggacgaactgtataaaggcagcggcggcacctaaggatcc

SEQ ID NO: 16 - DNA, 109 bp, Artificial Sequence
  Tag insert sequence
ccatgggtctgaacgacatcttcgaggcgcaaaaaattgagtggcacgaggagaacctgtacttccagggtcaccatcatcaccatcatatgcgtaagggcgaggaact

SEQ ID NO: 17 - DNA, 203 bp, Artificial Sequence
  GFP10-11
ggcgtaatacgactcactatagggttaactttaagaaggagatatacatatggacctgccggacgaccactacctgtctacccagaccatcctgctgaaagacctgaacgaaaaacgtgaccacatggttctgctggaatacgttaccgcggcgggtatcaccgacgcgtctggctctggctctggctctggctctaaaaaaa

SEQ ID NO: 18 - DNA, 140 bp, Artificial Sequence
  GFP10
ggcgtaatacgactcactatagggttaactttaagaaggagatatacatatggacctgccggacgaccactacctgtctacccagaccatcctgctgaaagacctgaacggctctggctctggctctggctctaaaaaaa

SEQ ID NO: 19 - DNA, 146 bp, Artificial Sequence
  GFP11
ggcgtaatacgactcactatagggttaactttaagaaggagatatacatatggaaaaacgtgatcatatggtgctgctggaatatgtgaccgcggcgggcattaccgatgcgtctggctctggctctggctctggctctaaaaaaa

SEQ ID NO: 20 - DNA, 117 bp, Artificial Sequence
  Rapamycin-nucleic acid
gtaatacgactcactatagggttaactttaagaaggagatatacatatgcagtttatgttttaggagattctgaggccgaccggcaccggcaccggcgatagggcggcggggacaaa

SEQ ID NO: 21 - DNA, 450 bp, Artificial Sequence
  Hisx6-FKBP12-Link12-GFP11
atgcaccaccaccaccaccacatgggcgtccaagtcgaaacgatcagtccgggcgatggccgtaccttcccgaaacgcggtcaaacgtgcgtggttcattataccggcatgctggaagatggtaaaaaatttgatagctctcgtgaccgcaacaaaccgtttaaattcatgctgggcaaacaggaagtgattcgtggctgggaagaaggtgttgcacagatgagcgtcggtcaacgcgctaaactgaccatcagtccggattatgcgtacggtgccacgggccatccgggtattatcccgccgcacgcaaccctggtctttgacgtggaactgctgaaactggaaggcggtggcggttcaggcggtggctcgggtggcagtacgtccgaaaaacgcgatcacatggttctgctggaatatgtcacggctgcgggtatcaccgatgcttcg

SEQ ID NO: 22 - DNA, 390 bp, Artificial Sequence
  GFP10-Link12-FRB-Hisx6
atggacctgccggacaatcactatctgagtacgcaaacgatcctgctgaaagacctgaacgatgttggtggtggtggctctggcggtggcagcggcggttctgaaatgtggcatgaaggtctggaagaagcaagccgtctgtattttggcgaacgcaacgtgaaaggcatgttcgaagttctggaaccgctgcacgctatgatggaacgtggcccgcagaccctgaaagaaacgagttttaaccaagcgtatggtcgtgatctgatggaagcccaggaatggtgccgcaaatacatgaaatccggcaatgtcaaagacctgacccaagcctgggacctgtattaccatgtctttcgtcgcatctctaaacaacaccatcatcatcaccat

SEQ ID NO: 23 - DNA, 359 bp, Artificial Sequence
  SNAP(N) whole_DNA
ggcgtaatacgactcactatagggttaactttaataaggagatataaatatggacaaagactgcgaaatgaagcgcaccaccctggatagccctctgggcaagctggaactgtctgggtgcgaacagggcctgcaccgtatcatcttcctgggcaaaggaacatctgccgccgacgccgtggaagtgcctgccccagccgccgtgctgggcggaccagagccactgatgcaggccaccgcctggctcaacgcctactttcaccagcctgaggccatcgaggagttccctgtgccagccctgcaccacccagtgttccagcagggctctggctctggctctggctctggctctaaaaaaa

SEQ ID NO: 24 - DNA, 404 bp, Artificial Sequence
  SNAP(C) whole_DNA
ggcgtaatacgactcactatagggttaactttaataaggagatataaatatggtcgacgagagctttacccgccaggtgctgtggaaactgctgaaagtggtgaagttcggagaggtcatcagctacagccacctggccgccctggccggcaatcccgccgccaccgccgccgtgaaaaccgccctgagcggaaatcccgtgcccattctgatcccctgccaccgggtggtgcagggcgacctggacgtggggggctacgagggcgggctcgccgtgaaagagtggctgctggcccacgagggccacagactgggcaagcctgggctgggtcctgcaggcggatccgcgtttaaactcgaggttaatggctctggctctggctctggctctggctctaaaaaaa

SEQ ID NO: 25 - DNA, 668 bp, Artificial Sequence
  SNAP(full) whole_DNA
ggcgtaatacgactcactatagggttaactttaataaggagatataaatatggacaaagactgcgaaatgaagcgcaccaccctggatagccctctgggcaagctggaactgtctgggtgcgaacagggcctgcaccgtatcatcttcctgggcaaaggaacatctgccgccgacgccgtggaagtgcctgccccagccgccgtgctgggcggaccagagccactgatgcaggccaccgcctggctcaacgcctactttcaccagcctgaggccatcgaggagttccctgtgccagccctgcaccacccagtgttccagcaggagagctttacccgccaggtgctgtggaaactgctgaaagtggtgaagttcggagaggtcatcagctacagccacctggccgccctggccggcaatcccgccgccaccgccgccgtgaaaaccgccctgagcggaaatcccgtgcccattctgatcccctgccaccgggtggtgcagggcgacctggacgtggggggctacgagggcgggctcgccgtgaaagagtggctgctggcccacgagggccacagactgggcaagcctgggctgggtcctgcaggcggatccgcgtttaaactcgaggttaatggctctggctctggctctggctctggctctaaaaaaa

SEQ ID NO: 26 - DNA, 194 bp, Artificial Sequence
  UbNter_DNA
ggcgtaatacgactcactatagggttaactttaagaaggagatatacatatgatgcagatcttcgtgaagaccctgaccggcaagaccgccactctggaggtggagcccagtgacaccatcgaaaatgtgaaggccaagatccaagataaagaaggcatccccggctctggctctggctctggctctaaaaaaa

SEQ ID NO: 27 - DNA, 209 bp, Artificial Sequence
  UbCter_DNA
ggcgtaatacgactcactatagggttaactttaagaaggagatatacatatgggcatcccccccgaccagcagaggctcatctttgcaggcaagcagctggaagatggccgcactctttctgactacaacatccagaaagagtcgaccctgcacctggtcctgcgcctgaggggtggcggctctggctctggctctggctctaaaaaaa

SEQ ID NO: 28 - DNA, 332 bp, Artificial Sequence
  UbI13A full_DNA
ggcgtaatacgactcactatagggttaactttaagaaggagatatacatatgatgcagatcttcgtgaagaccctgaccggcaagaccgccactctggaggtggagcccagtgacaccatcgaaaatgtgaaggccaagatccaagataaagaaggcatccccggctctggctctggcatcccccccgaccagcagaggctcatctttgcaggcaagcagctggaagatggccgcactctttctgactacaacatccagaaagagtcgaccctgcacctggtcctgcgcctgaggggtggcggctctggctctggctctggctctaaaaaaa

SEQ ID NO: 29 - RNA, 182 nt, Artificial Sequence
  GFP10-11
ggguuaacuuuaagaaggagauauacauauggaccugccggacgaccacuaccugucuacccagaccauccugcugaaagaccugaacgaaaaacgugaccacaugguucugcuggaauacguuaccgcggcggguaucaccgacgcgucuggcucuggcucuggcucuggcucuaaaaaaa

SEQ ID NO: 30 - RNA, 119 nt, Artificial Sequence
  GFP10
ggguuaacuuuaagaaggagauauacauauggaccugccggacgaccacuaccugucuacccagaccauccugcugaaagaccugaacggcucuggcucuggcucuggcucuaaaaaaa

SEQ ID NO: 31 - RNA, 125 nt, Artificial Sequence
  GFP11
ggguuaacuuuaagaaggagauauacauauggaaaaacgugaucauauggugcugcuggaauaugugaccgcggcgggcauuaccgaugcgucuggcucuggcucuggcucuggcucuaaaaaaa

SEQ ID NO: 32 - RNA, 99 nt, Artificial Sequence
  Rapamycin-nucleic acid
ggguuaacuuuaagaaggagauauacauaugcaguuuauguuuuaggagauucugaggccgaccggcaccggcaccggcgauagggcggcggggacaaa

SEQ ID NO: 33 - RNA, 338 nt, Artificial Sequence
  SNAP(N) whole_mRNA
ggguuaacuuuaauaaggagauauaaauauggacaaagacugcgaaaugaagcgcaccacccuggauagcccucugggcaagcuggaacugucugggugcgaacagggccugcaccguaucaucuuccugggcaaaggaacaucugccgccgacgccguggaagugccugccccagccgccgugcugggcggaccagagccacugaugcaggccaccgccuggcucaacgccuacuuucaccagccugaggccaucgaggaguucccugugccagcccugcaccacccaguguuccagcagggcucuggcucuggcucuggcucuggcucuaaaaaaa

SEQ ID NO: 34 - RNA, 383 nt, Artificial Sequence
  SNAP(C) whole_mRNA
ggguuaacuuuaauaaggagauauaaauauggucgacgagagcuuuacccgccaggugcuguggaaacugcugaaaguggugaaguucggagaggucaucagcuacagccaccuggccgcccuggccggcaaucccgccgccaccgccgccgugaaaaccgcccugagcggaaaucccgugcccauucugauccccugccaccggguggugcagggcgaccuggacguggggggcuacgagggcgggcucgccgugaaagaguggcugcuggcccacgagggccacagacugggcaagccugggcuggguccugcaggcggauccgcguuuaaacucgagguuaauggcucuggcucuggcucuggcucuggcucuaaaaaaa

SEQ ID NO: 35 - RNA, 647 nt, Artificial Sequence
  SNAP(full) whole_mRNA
ggguuaacuuuaauaaggagauauaaauauggacaaagacugcgaaaugaagcgcaccacccuggauagcccucugggcaagcuggaacugucugggugcgaacagggccugcaccguaucaucuuccugggcaaaggaacaucugccgccgacgccguggaagugccugccccagccgccgugcugggcggaccagagccacugaugcaggccaccgccuggcucaacgccuacuuucaccagccugaggccaucgaggaguucccugugccagcccugcaccacccaguguuccagcaggagagcuuuacccgccaggugcuguggaaacugcugaaaguggugaaguucggagaggucaucagcuacagccaccuggccgcccuggccggcaaucccgccgccaccgccgccgugaaaaccgcccugagcggaaaucccgugcccauucugauccccugccaccggguggugcagggcgaccuggacguggggggcuacgagggcgggcucgccgugaaagaguggcugcuggcccacgagggccacagacugggcaagccugggcuggguccugcaggcggauccgcguuuaaacucgagguuaauggcucuggcucuggcucuggcucuggcucuaaaaaaa

SEQ ID NO: 36 - RNA, 173 nt, Artificial Sequence
  UbNter_mRNA
ggguuaacuuuaagaaggagauauacauaugaugcagaucuucgugaagacccugaccggcaagaccgccacucuggagguggagcccagugacaccaucgaaaaugugaaggccaagauccaagauaaagaaggcauccccggcucuggcucuggcucuggcucuaaaaaaa

SEQ ID NO: 37 - RNA, 188 nt, Artificial Sequence
  UbCter_mRNA
ggguuaacuuuaagaaggagauauacauaugggcaucccccccgaccagcagaggcucaucuuugcaggcaagcagcuggaagauggccgcacucuuucugacuacaacauccagaaagagucgacccugcaccugguccugcgccugagggguggcggcucuggcucuggcucuggcucuaaaaaaa

SEQ ID NO: 38 - RNA, 311 nt, Artificial Sequence
  UbI13A full_mRNA
ggguuaacuuuaagaaggagauauacauaugaugcagaucuucgugaagacccugaccggcaagaccgccacucuggagguggagcccagugacaccaucgaaaaugugaaggccaagauccaagauaaagaaggcauccccggcucuggcucuggcaucccccccgaccagcagaggcucaucuuugcaggcaagcagcuggaagauggccgcacucuuucugacuacaacauccagaaagagucgacccugcaccugguccugcgccugagggguggcggcucuggcucuggcucuggcucuaaaaaaa

SEQ ID NO: 39 - protein, 51 aa, Artificial Sequence
  GFP10-GFP11-GS4
MDLPDDHYLSTQTILLKDLNEKRDHMVLLEYVTAAGITDASGSGSGSGSKK

SEQ ID NO: 40 - protein, 30 aa, Artificial Sequence
  GFP10-GS4
MDLPDDHYLSTQTILLKDLNGSGSGSGSKK

SEQ ID NO: 41 - protein, 32 aa, Artificial Sequence
  GFP11-GS4
MEKRDHMVLLEYVTAAGITDASGSGSGSGSKK

SEQ ID NO: 42 - protein, 103 aa, Artificial Sequence
  splitSNAP (N)-GS5
MDKDCEMKRTTLDSPLGKLELSGCEQGLHRIIFLGKGTSAADAVEVPAPAAVLGGPEPLMQATAWLNAYFHQPEAIEEFPVPALHHPVFQQGSGSGSGSGSKK

SEQ ID NO: 43 - protein, 118 aa, Artificial Sequence
  SNAP (C)-GS5
MVDESFTRQVLWKLLKVVKFGEVISYSHLAALAGNPAATAAVKTALSGNPVPILIPCHRVVQGDLDVGGYEGGLAVKEWLLAHEGHRLGKPGLGPAGGSAFKLEVNGSGSGSGSGSKK

SEQ ID NO: 44 - protein, 206 aa, Artificial Sequence
  SNAP (full)-GS5
MDKDCEMKRTTLDSPLGKLELSGCEQGLHRIIFLGKGTSAADAVEVPAPAAVLGGPEPLMQATAWLNAYFHQPEAIEEFPVPALHHPVFQQESFTRQVLWKLLKVVKFGEVISYSHLAALAGNPAATAAVKTALSGNPVPILIPCHRVVQGDLDVGGYEGGLAVKEWLLAHEGHRLGKPGLGPAGGSAFKLEVNGSGSGSGSGSKK

SEQ ID NO: 45 - protein, 48 aa, Artificial Sequence
  splitUb (N)-GS4
MMQIFVKTLTGKTATLEVEPSDTIENVKAKIQDKEGIPGSGSGSGSKK

SEQ ID NO: 46 - protein, 53 aa, Artificial Sequence
  splitUb (C)-GS4
MGIPPDQQRLIFAGKQLEDGRTLSDYNIQKESTLHLVLRLRGGGSGSGSGSKK

SEQ ID NO: 47 - protein, 94 aa, Artificial Sequence
  splitUb (N-C)-GS4
MMQIFVKTLTGKTATLEVEPSDTIENVKAKIQDKEGIPGSGSGIPPDQQRLIFAGKQLEDGRTLSDYNIQKESTLHLVLRLRGGGSGSGSGSKK

SEQ ID NO: 48 - protein, 233 aa, Artificial Sequence
  Avi-Tev-His-GFP1-9
MGLNDIFEAQKIEWHEENLYFQGHHHHHHGGSSSKGEELFTGVVPILVELDGDVNGHKFSVRGEGEGDATIGKLTLKFISTTGKLPVPWPTLVTTLTYGVQAFSRYPDHMKRHDFFKSAMPEGYVQERTISFKDDGKYKTRAVVKFEGDTLVNRIELKGTDFKEDGNILGHKLEYNFNSHNVYITADKQKNGIKANFTVRHNVEDGSVQLADHYQQNTPIGDGTRGSGSIEGR

SEQ ID NO: 49 - DNA, 320 bp, Artificial Sequence
  Kpep-UbNter_DNA
gtaatacgactcactatagggttaactttaagaaggagatatacatatgaaagtgagcgcgctgaaagaaaacgtgagcgccctgaaagaaaaagtgagcgcgctgaccgaaaaagtgagcgcgctgaaagagaaagtgagcgcgctgaaagaaggctctggctctggctctggctctatgcagatcttcgtgaagaccctgaccggcaagaccgccactctggaggtggagcccagtgacaccatcgaaaatgtgaaggccaagatccaagataaagaaggcatccccggctctggctctggctctggctctaaaaaaa

SEQ ID NO: 50 - DNA, 320 bp, Artificial Sequence
  Epep-UbNter_DNA
gtaatacgactcactatagggttaactttaagaaggagatatacatatgaaagtgagcgcgctggaaaacgaagtgagcgcgctggaaaaagaagtgagcgtgctggaaaaagaagtgagcgcgctggaaaaagaagtgcgcgcgctggaaaaaggctctggctctggctctggctctatgcagatcttcgtgaagaccctgaccggcaagaccgccactctggaggtggagcccagtgacaccatcgaaaatgtgaaggccaagatccaagataaagaaggcatccccggctctggctctggctctggctctaaaaaaa

SEQ ID NO: 51 - DNA, 338 bp, Artificial Sequence
  Epep-UbCter_DNA
ggcgtaatacgactcactatagggttaactttaagaaggagatatacatatgggcatcccccccgaccagcagaggctcatctttgcaggcaagcagctggaagatggccgcactctttctgactacaacatccagaaagagtcgaccctgcacctggtcctgcgcctgaggggtggcggctctggctctggctctggctctaaagtgagcgcgctggaaaacgaagtgagcgcgctggaaaaagaagtgagcgtgctggaaaaagaagtgagcgcgctggaaaaagaagtgcgcgcgctggaaaaaggctctggctctggctctggctctaaaaaaa

SEQ ID NO: 52 - RNA, 302 nt, Artificial Sequence
  Kpep-UbNter_mRNA
ggguuaacuuuaagaaggagauauacauaugaaagugagcgcgcugaaagaaaacgugagcgcccugaaagaaaaagugagcgcgcugaccgaaaaagugagcgcgcugaaagagaaagugagcgcgcugaaagaaggcucuggcucuggcucuggcucuaugcagaucuucgugaagacccugaccggcaagaccgccacucuggagguggagcccagugacaccaucgaaaaugugaaggccaagauccaagauaaagaaggcauccccggcucuggcucuggcucuggcucuaaaaaaa

SEQ ID NO: 53 - RNA, 302 nt, Artificial Sequence
  Epep-UbNter_mRNA
ggguuaacuuuaagaaggagauauacauaugaaagugagcgcgcuggaaaacgaagugagcgcgcuggaaaaagaagugagcgugcuggaaaaagaagugagcgcgcuggaaaaagaagugcgcgcgcuggaaaaaggcucuggcucuggcucuggcucuaugcagaucuucgugaagacccugaccggcaagaccgccacucuggagguggagcccagugacaccaucgaaaaugugaaggccaagauccaagauaaagaaggcauccccggcucuggcucuggcucuggcucuaaaaaaa

SEQ ID NO: 54 - RNA, 317 nt, Artificial Sequence
  Epep-UbCter_mRNA
ggguuaacuuuaagaaggagauauacauaugggcaucccccccgaccagcagaggcucaucuuugcaggcaagcagcuggaagauggccgcacucuuucugacuacaacauccagaaagagucgacccugcaccugguccugcgccugagggguggcggcucuggcucuggcucuggcucuaaagugagcgcgcuggaaaacgaagugagcgcgcuggaaaaagaagugagcgugcuggaaaaagaagugagcgcgcuggaaaaagaagugcgcgcgcuggaaaaaggcucuggcucuggcucuggcucuaaaaaaa

SEQ ID NO: 55 - protein, 91 aa, Artificial Sequence
  Kpep-splitUb(N)-GS4
MKVSALKENVSALKEKVSALTEKVSALKEKVSALKEGSGSGSGSMQIFVKTLTGKTATLEVEPSDTIENVKAKIQDKEGIPGSGSGSGSKK

SEQ ID NO: 56 - protein, 91 aa, Artificial Sequence
  Epep-splitUb(N)-GS4
MKVSALENEVSALEKEVSVLEKEVSALEKEVRALEKGSGSGSGSMQIFVKTLTGKTATLEVEPSDTIENVKAKIQDKEGIPGSGSGSGSKK

SEQ ID NO: 57 - protein, 96 aa, Artificial Sequence
  Epep-splitUb(C)-GS4
MGIPPDQQRLIFAGKQLEDGRTLSDYNIQKESTLHLVLRLRGGGSGSGSGSKVSALENEVSALEKEVSVLEKEVSALEKEVRALEKGSGSGSGSKK

SEQ ID NO: 58 - DNA, 533 bp, Artificial Sequence
  Avi-His-splitNanoluc1-8
ccatgggcctgaacgatatttttgaagcgcagaagattgagtggcacgaacaccatcatcatcatcacggtggtagcagcgtgttcaccctggaggactttgttggcgattgggaacagaccgcggcgtacaacctggaccaggtgctggagcaaggtggcgttagcagcctgctgcagaacctggcggtgagcgttaccccgatccaacgtattgttcgtagcggcgagaacgcgctgaagatcgacattcacgtgatcattccgtatgaaggcctgagcgcggatcagatggcgcaaatcgaggaagtgttcaaggtggtttacccggttgacgatcaccactttaaagtgatcctgccgtatggtaccctggtgattgacggcgttaccccgaacatgctgaactacttcggtcgtccgtatgaaggcatcgcggtttttgatggtaagaaaattaccgttaccggcaccctgtggaacggcaacaagattattgacgaacgcctgattaccccggactaatgaggatcc

SEQ ID NO: 59 - DNA, 200 bp, Artificial Sequence
  Nanoluc9-10
ggcgtaatacgactcactatagggttaactttaagaaggagatatacatatgggcagcatgctgtttcgtgtgaccattaacagcggcggcggcagcggcggcggcggcagcggcgtgagcggctggcgtctgtttaaaaaaattagcggttctggttctggttctggttctgaaaacctgtattttcagggcaaaaaaa

SEQ ID NO: 60 - DNA, 137 bp, Artificial Sequence
  Nanoluc-9
ggcgtaatacgactcactatagggttaactttaagaaggagatatacatatgggcagcatgctgtttcgtgtgaccattaacagcggttctggttctggttctggttctgaaaacctgtattttcagggcaaaaaaa

SEQ ID NO: 61 - DNA, 137 bp, Artificial Sequence
  Nanoluc-10
ggcgtaatacgactcactatagggttaactttaagaaggagatatacatatggtgagcggctggcgtctgtttaaaaaaattagcggttctggttctggttctggttctgaaaacctgtattttcagggcaaaaaaa

SEQ ID NO: 62 - RNA, 179 nt, Artificial Sequence
  Nanoluc9-10
ggguuaacuuuaagaaggagauauacauaugggcagcaugcuguuucgugugaccauuaacagcggcggcggcagcggcggcggcggcagcggcgugagcggcuggcgucuguuuaaaaaaauuagcgguucugguucugguucugguucugaaaaccuguauuuucagggcaaaaaaa

SEQ ID NO: 63 - RNA, 116 nt, Artificial Sequence
  Nanoluc-9
ggguuaacuuuaagaaggagauauacauaugggcagcaugcuguuucgugugaccauuaacagcgguucugguucugguucugguucugaaaaccuguauuuucagggcaaaaaaa

SEQ ID NO: 64 - RNA, 116 nt, Artificial Sequence
  Nanoluc-10
ggguuaacuuuaagaaggagauauacauauggugagcggcuggcgucuguuuaaaaaaauuagcgguucugguucugguucugguucugaaaaccuguauuuucagggcaaaaaaa

SEQ ID NO: 65 - protein, 50 aa, Artificial Sequence
  SplitNanoluc9-10-GS4-TEV
MGSMLFRVTINSGGGSGGGGSGVSGWRLFKKISGSGSGSGSENLYFQGKK

SEQ ID NO: 66 - protein, 29 aa, Artificial Sequence
  SplitNanoluc-9-GS4-TEV
MGSMLFRVTINSGSGSGSGSENLYFQGKK

SEQ ID NO: 67 - protein, 29 aa, Artificial Sequence
  SplitNanoluc-10-GS4-TEV
MVSGWRLFKKISGSGSGSGSENLYFQGKK

SEQ ID NO: 68 - DNA, 28 bp, Artificial Sequence
  Nanoluc_qPCR_Rvprimer
tttttttgccctgaaaatacaggttttc

SEQ ID NO: 69 - DNA, 23 bp, Artificial Sequence
  Fw primer for #13Rapa_F5
gatatacatatgcagtttatgtt

SEQ ID NO: 70 - DNA, 21 bp, Artificial Sequence
  Rv primer for #13Rapa_R4
ggtcggcctcagaatctccta

SEQ ID NO: 71 - protein, 231 aa, Artificial Sequence
  GFP full
MSKGEELFTGVVPILVELDGDVNGHKFSVRGEGEGDATIGKLTLKFISTTGKLPVPWPTLVTTLTYGVQAFSRYPDHMKRHDFFKSAMPEGYVQERTISFKDDGKYKTRAVVKFEGDTLVNRIELKGTDFKEDGNILGHKLEYNFNSHNVYITADKQKNGIKANFTVRHNVEDGSVQLADHYQQNTPIGDGDLPDDHYLSTQTILLKDLNEKRDHMVLLEYVTAAGITDAS

SEQ ID NO: 72 - protein, 191 aa, Artificial Sequence
  GFP1-9
MSKGEELFTGVVPILVELDGDVNGHKFSVRGEGEGDATIGKLTLKFISTTGKLPVPWPTLVTTLTYGVQAFSRYPDHMKRHDFFKSAMPEGYVQERTISFKDDGKYKTRAVVKFEGDTLVNRIELKGTDFKEDGNILGHKLEYNFNSHNVYITADKQKNGIKANFTVRHNVEDGSVQLADHYQQNTPIGDG

SEQ ID NO: 73 - protein, 19 aa, Artificial Sequence
  GFP10
DLPDDHYLSTQTILLKDLN

SEQ ID NO: 74 - protein, 21 aa, Artificial Sequence
  GFP11
EKRDHMVLLEYVTAAGITDAS

SEQ ID NO: 75 - protein, 76 aa, Artificial Sequence
  Ubiquitin full
MQIFVKTLTGKTATLEVEPSDTIENVKAKIQDKEGIPPDQQRLIFAGKQLEDGRTLSDYNIQKESTLHLVLRLRGG

SEQ ID NO: 76 - protein, 37 aa, Artificial Sequence
  splitUb (N)
MQIFVKTLTGKTATLEVEPSDTIENVKAKIQDKEGIP

SEQ ID NO: 77 - protein, 42 aa, Artificial Sequence
  splitUb (C)
GIPPDQQRLIFAGKQLEDGRTLSDYNIQKESTLHLVLRLRGG

SEQ ID NO: 78 - protein, 170 aa, Artificial Sequence
  Nanoluc full
MVFTLEDFVGDWEQTAAYNLDQVLEQGGVSSLLQNLAVSVTPIQRIVRSGENALKIDIHVIIPYEGLSADQMAQIEEVFKVVYPVDDHHFKVILPYGTLVIDGVTPNMLNYFGRPYEGIAVFDGKKITVTGTLWNGNKIIDERLITPDGSMLFRVTINSVSGWRLFKKIS

SEQ ID NO: 79 - protein, 148 aa, Artificial Sequence
  SplitNanoluc1-8
MVFTLEDFVGDWEQTAAYNLDQVLEQGGVSSLLQNLAVSVTPIQRIVRSGENALKIDIHVIIPYEGLSADQMAQIEEVFKVVYPVDDHHFKVILPYGTLVIDGVTPNMLNYFGRPYEGIAVFDGKKITVTGTLWNGNKIIDERLITPD

SEQ ID NO: 80 - protein, 11 aa, Artificial Sequence
  SplitNanoluc-9
GSMLFRVTINS

SEQ ID NO: 81 - protein, 11 aa, Artificial Sequence
  SplitNanoluc-10
VSGWRLFKKIS

SEQ ID NO: 82 - protein, 194 aa, Artificial Sequence
  SNAP (full)
MDKDCEMKRTTLDSPLGKLELSGCEQGLHRIIFLGKGTSAADAVEVPAPAAVLGGPEPLMQATAWLNAYFHQPEAIEEFPVPALHHPVFQQESFTRQVLWKLLKVVKFGEVISYSHLAALAGNPAATAAVKTALSGNPVPILIPCHRVVQGDLDVGGYEGGLAVKEWLLAHEGHRLGKPGLGPAGGSAFKLEVN

SEQ ID NO: 83 - protein, 91 aa, Artificial Sequence
  SplitSNAP (N)
MDKDCEMKRTTLDSPLGKLELSGCEQGLHRIIFLGKGTSAADAVEVPAPAAVLGGPEPLMQATAWLNAYFHQPEAIEEFPVPALHHPVFQQ

SEQ ID NO: 84 - protein, 105 aa, Artificial Sequence
  SplitSNAP (C)
VDESFTRQVLWKLLKVVKFGEVISYSHLAALAGNPAATAAVKTALSGNPVPILIPCHRVVQGDLDVGGYEGGLAVKEWLLAHEGHRLGKPGLGPAGGSAFKLEVN

SEQ ID NO: 85 - protein, 173 aa, Artificial Sequence
  Avi-His-spNluc1-8
MGLNDIFEAQKIEWHEHHHHHHGGSSVFTLEDFVGDWEQTAAYNLDQVLEQGGVSSLLQNLAVSVTPIQRIVRSGENALKIDIHVIIPYEGLSADQMAQIEEVFKVVYPVDDHHFKVILPYGTLVIDGVTPNMLNYFGRPYEGIAVFDGKKITVTGTLWNGNKIIDERLITPD

SEQ ID NO: 86 - protein, 150 aa, Artificial Sequence
  Hisx6-FKBP12-Link12-GFP11
MHHHHHHMGVQVETISPGDGRTFPKRGQTCVVHYTGMLEDGKKFDSSRDRNKPFKFMLGKQEVIRGWEEGVAQMSVGQRAKLTISPDYAYGATGHPGIIPPHATLVFDVELLKLEGGGGSGGGSGGSTSEKRDHMVLLEYVTAAGITDAS

SEQ ID NO: 87 - protein, 130 aa, Artificial Sequence
  GFP10-Link12-FRB-Hisx6
MDLPDNHYLSTQTILLKDLNDVGGGGSGGGSGGSEMWHEGLEEASRLYFGERNVKGMFEVLEPLHAMMERGPQTLKETSFNQAYGRDLMEAQEWCRKYMKSGNVKDLTQAWDLYYHVFRRISKQHHHHHH

SEQ ID NO: 88 - protein, 4 aa, Artificial Sequence
  GS linker
GGSS

SEQ ID NO: 89 - protein, 4 aa, Artificial Sequence
  GS linker
GGGS

SEQ ID NO: 90 - protein, 4 aa, Artificial Sequence
  GS linker
SGGG

SEQ ID NO: 91 - protein, 4 aa, Artificial Sequence
  GS linker
GSGS

SEQ ID NO: 92 - protein, 5 aa, Artificial Sequence
  GS linker
GGGGS

SEQ ID NO: 93 - protein, 5 aa, Artificial Sequence
  GS linker
SGGGG

SEQ ID NO: 94 - protein, 6 aa, Artificial Sequence
  GS linker
GGGGGS

SEQ ID NO: 95 - protein, 6 aa, Artificial Sequence
  GS linker
SGGGGG

SEQ ID NO: 96 - protein, 7 aa, Artificial Sequence
  GS linker
GGGGGGS

SEQ ID NO: 97 - protein, 7 aa, Artificial Sequence
  GS linker
SGGGGGG

SEQ ID NO: 98 - DNA, 17 bp, Artificial Sequence
  Annealing seq. for Rapamycin-nucleic acid prep.
cccgtccccgccgccct

SEQ ID NO: 99 - DNA, 38 bp, Artificial Sequence
  SNAP_qPCR_Fw
gtaatacgactcactatagggttaactttaataaggag

SEQ ID NO: 100 - protein, 233 aa, Artificial Sequence
  KRAS-FLAGSorHisTEV-Bio
MTEYKLVVVGADGVGKSALTIQLIQNHFVDEYDPTIEDSYRKQVVIDGETCLLDILDTAGQEEYSAMRDQYMRTGEGFLCVFAINNTKSFEDIHHYREQIKRVKDSEDVPMVLVGNKCDLPSRTVDTKQAQDLARSYGIPFIETSAKTRQGVDDAFYTLVREIRKHKEKMSKDGGSSDYKDDDDKGGSSLPMTGGGGSSHHHHHHSSGENLYFQGSGGGLNDIFEAQKIEWHE

SEQ ID NO: 101 - protein, 205 aa, Artificial Sequence
  HAT-KRAS-nonbio
MKDHLIHNVHKEEHAHAHSSGSLVPRGSSGGSTEYKLVVVGADGVGKSALTIQLIQNHFVDEYDPTIEDSYRKQVVIDGETCLLDILDTAGQEEYSAMRDQYMRTGEGFLCVFAINNTKSFEDIHHYREQIKRVKDSEDVPMVLVGNKCDLPSRTVDTKQAQDLARSYGIPFIETSAKTRQGVDDAFYTLVREIRKHKEKMSKDG

SEQ ID NO: 102 - protein, 258 aa, Artificial Sequence
  GST-HisTEV-Bio
MSPILGYWKIKGLVQPTRLLLEYLEEKYEEHLYERDEGDKWRNKKFELGLEFPNLPYYIDGDVKLTQSMAIIRYIADKHNMLGGCPKERAEISMLEGAVLDIRYGVSRIAYSKDFETLKVDFLSKLPEMLKMFEDRLCHKTYLNGDHVTHPDFMLYDALDVVLYMDPMCLDAFPKLVCFKKRIEAIPQIDKYLKSSKYIAWPLQGWQATFGGGDHPPKSDGGSSHHHHHHSSGENLYFQGSGGGLNDIFEAQKIEWHE

SEQ ID NO: 103 - protein, 258 aa, Artificial Sequence; identical to SEQ ID NO: 102
  GST-HisTEVAvi

SEQ ID NO: 104 - protein, 254 aa, Artificial Sequence
  GST-SrtAHis
MSPILGYWKIKGLVQPTRLLLEYLEEKYEEHLYERDEGDKWRNKKFELGLEFPNLPYYIDGDVKLTQSMAIIRYIADKHNMLGGCPKERAEISMLEGAVLDIRYGVSRIAYSKDFETLKVDFLSKLPEMLKMFEDRLCHKTYLNGDHVTHPDFMLYDALDVVLYMDPMCLDAFPKLVCFKKRIEAIPQIDKYLKSSKYIAWPLQGWQATFGGGDHPPKSDGGSSDYKDDDDKGGSSLPMTGGGGSSHHHHHHHH

SEQ ID NO: 105 - protein, 156 aa, Artificial Sequence
  eSrtA
MQAKPQIPKDKSKVAGYIEIPDADIKEPVYPGPATREQLNRGVSFAEENESLDDQNISIAGHTFIDRPNYQFTNLKAAKKGSMVYFKVGNETRKYKMTSIRNVKPTAVEVLDEQKGKDKQLTLITCDDYNEETGVWETRKIFVATEVKLEHHHHHH

SEQ ID NO: 106 - protein, 35 aa, Artificial Sequence
  Sor-sp11-L12
GGGGSGGGSGGSTSEKRDHMVLLEYVTAAGITDAS

SEQ ID NO: 107 - protein, 32 aa, Artificial Sequence
  Sor-sp10-12
GGGGSGGGSGGSMDLPDDHYLSTQTILLKDLN

SEQ ID NO: 108 - protein, 228 aa, Artificial Sequence
  KRAS-sp11
MTEYKLVVVGADGVGKSALTIQLIQNHFVDEYDPTIEDSYRKQVVIDGETCLLDILDTAGQEEYSAMRDQYMRTGEGFLCVFAINNTKSFEDIHHYREQIKRVKDSEDVPMVLVGNKCDLPSRTVDTKQAQDLARSYGIPFIETSAKTRQGVDDAFYTLVREIRKHKEKMSKDGGSSDYKDDDDKGGSSLPMTGGGGSGGGSGGSTSEKRDHMVLLEYVTAAGITDAS

SEQ ID NO: 109 - protein, 225 aa, Artificial Sequence
  KRAS-sp10
MTEYKLVVVGADGVGKSALTIQLIQNHFVDEYDPTIEDSYRKQVVIDGETCLLDILDTAGQEEYSAMRDQYMRTGEGFLCVFAINNTKSFEDIHHYREQIKRVKDSEDVPMVLVGNKCDLPSRTVDTKQAQDLARSYGIPFIETSAKTRQGVDDAFYTLVREIRKHKEKMSKDGGSSDYKDDDDKGGSSLPMTGGGGSGGGSGGSMDLPDDHYLSTQTILLKDLN

SEQ ID NO: 110 - protein, 272 aa, Artificial Sequence
  GST-sp10
MSPILGYWKIKGLVQPTRLLLEYLEEKYEEHLYERDEGDKWRNKKFELGLEFPNLPYYIDGDVKLTQSMAIIRYIADKHNMLGGCPKERAEISMLEGAVLDIRYGVSRIAYSKDFETLKVDFLSKLPEMLKMFEDRLCHKTYLNGDHVTHPDFMLYDALDVVLYMDPMCLDAFPKLVCFKKRIEAIPQIDKYLKSSKYIAWPLQGWQATFGGGDHPPKSDGGSSDYKDDDDKGGSSLPMTGGGGSGGGSGGSMDLPDDHYLSTQTILLKDLN

SEQ ID NO: 111 - DNA, 107 bp, Artificial Sequence
  DNA library
  misc_feature (50)..(52): nnn = ttt, ttg, ctt, ctg, att, atg, gtt, gtg, tct, tcg, ccg, act, gct, tac, cat, cag, aac, gat, gag, tgc, tgg, cgt, cgg, agt, agg, or ggt
  misc_feature (53)..(55): nnn = ttt, ttg, ctt, ctg, att, atg, gtt, gtg, tct, tcg, ccg, act, gct, tac, cat, cag, aac, gat, gag, tgc, tgg, cgt, cgg, agt, agg, or ggt
  misc_feature (56)..(58): nnn = ttt, ttg, ctt, ctg, att, atg, gtt, gtg, tct, tcg, ccg, act, gct, tac, cat, cag, aac, gat, gag, tgc, tgg, cgt, cgg, agt, agg, or ggt
  misc_feature (59)..(61): nnn = ttt, ttg, ctt, ctg, att, atg, gtt, gtg, tct, tcg, ccg, act, gct, tac, cat, cag, aac, gat, gag, tgc, tgg, cgt, cgg, agt, agg, or ggt
  misc_feature (62)..(64): nnn = ttt, ttg, ctt, ctg, att, atg, gtt, gtg, tct, tcg, ccg, act, gct, tac, cat, cag, aac, gat, gag, tgc, tgg, cgt, cgg, agt, agg, or ggt
  misc_feature (65)..(67): nnn = ttt, ttg, ctt, ctg, att, atg, gtt, gtg, tct, tcg, ccg, act, gct, tac, cat, cag, aac, gat, gag, tgc, tgg, cgt, cgg, agt, agg, or ggt
  misc_feature (68)..(70): nnn = ttt, ttg, ctt, ctg, att, atg, gtt, gtg, tct, tcg, ccg, act, gct, tac, cat, cag, aac, gat, gag, tgc, tgg, cgt, cgg, agt, agg, or ggt
  misc_feature (71)..(73): nnn = ttt, ttg, ctt, ctg, att, atg, gtt, gtg, tct, tcg, ccg, act, gct, tac, cat, cag, aac, gat, gag, tgc, tgg, cgt, cgg, agt, agg, or ggt
  misc_feature (74)..(76): nnn = ttt, ttg, ctt, ctg, att, atg, gtt, gtg, tct, tcg, ccg, act, gct, tac, cat, cag, aac, gat, gag, tgc, tgg, cgt, cgg, agt, agg, or ggt
gtaatacgactcactatagggttaactttaataaggagatataaatatgnnnnnnnnnnnnnnnnnnnnnnnnnnntagccgaccggcaccggcaccggcaaaaaaa

SEQ ID NO: 112 - DNA, 38 bp, Artificial Sequence; identical to SEQ ID NO: 99
  qPCR primer_Fw

SEQ ID NO: 113 - DNA, 31 bp, Artificial Sequence
  qPCR primer_Rv
tttttttgccggtgccggtgccggtcggcta

SEQ ID NO: 114 - protein, 156 aa, Artificial Sequence
  FKBP-HisTEVAvi
MGVQVETISPGDGRTFPKRGQTCVVHYTGMLEDGKKFDSSRDRNKPFKFMLGKQEVIRGWEEGVAQMSVGQRAKLTISPDYAYGATGHPGIIPPHATLVFDVELLKLEGGSSLPMTGGGGSSHHHHHHSSGENLYFQGSGGGLNDIFEAQKIEWHE

SEQ ID NO: 115 - protein, 156 aa, Artificial Sequence; identical to SEQ ID NO: 114
  FKBP-SrtAHis

SEQ ID NO: 116 - protein, 5 aa, Artificial Sequence
  sortase recognition sequence
  misc_feature (3)..(3): Xaa can be any naturally occurring amino acid
LPXTG

SEQ ID NO: 117 - DNA, 39 bp, Artificial Sequence
  Fw-primer
gtaatacgactcactatagggttaactttaagaaggaga

SEQ ID NO: 118 - DNA, 43 bp, Artificial Sequence
  Rv-primer
tttgtccccgccgccctatcgccggtgccggtgccggtcggct

SEQ ID NO: 119 - DNA, 104 bp, Artificial Sequence
  v9case1 lib
  misc_feature (50)..(52): nnn = ttt, ttg, ctt, ctg, att, atg, gtt, gtg, tct, tcg, ccg, act, gct, tac, cat, cag, aac, gat, gag, tgc, tgg, cgt, cgg, agt, agg, or ggt
  misc_feature (53)..(55): nnn = ttt, ttg, ctt, ctg, att, atg, gtt, gtg, tct, tcg, ccg, act, gct, tac, cat, cag, aac, gat, gag, tgc, tgg, cgt, cgg, agt, agg, or ggt
  misc_feature (56)..(58): nnn = ttt, ttg, ctt, ctg, att, atg, gtt, gtg, tct, tcg, ccg, act, gct, tac, cat, cag, aac, gat, gag, tgc, tgg, cgt, cgg, agt, agg, or ggt
  misc_feature (59)..(61): nnn = ttt, ttg, ctt, ctg, att, atg, gtt, gtg, tct, tcg, ccg, act, gct, tac, cat, cag, aac, gat, gag, tgc, tgg, cgt, cgg, agt, agg, or ggt
  misc_feature (62)..(64): nnn = ttt, ttg, ctt, ctg, att, atg, gtt, gtg, tct, tcg, ccg, act, gct, tac, cat, cag, aac, gat, gag, tgc, tgg, cgt, cgg, agt, agg, or ggt
  misc_feature (65)..(67): nnn = ttt, ttg, ctt, ctg, att, atg, gtt, gtg, tct, tcg, ccg, act, gct, tac, cat, cag, aac, gat, gag, tgc, tgg, cgt, cgg, agt, agg, or ggt
  misc_feature (68)..(70): nnn = ttt, ttg, ctt, ctg, att, atg, gtt, gtg, tct, tcg, ccg, act, gct, tac, cat, cag, aac, gat, gag, tgc, tgg, cgt, cgg, agt, agg, or ggt
  misc_feature (71)..(73): nnn = ttt, ttg, ctt, ctg, att, atg, gtt, gtg, tct, tcg, ccg, act, gct, tac, cat, cag, aac, gat, gag, tgc, tgg, cgt, cgg, agt, agg, or ggt
gtaatacgactcactatagggttaactttaataaggagatataaatatgnnnnnnnnnnnnnnnnnnnnnnnntagccgaccggcaccggcaccggcaaaaaaa

SEQ ID NO: 120 - DNA, 120 bp, Artificial Sequence
  v7c1 ID45_9 (ATG)
  misc_feature (50)..(52): nnn = aac, act, agg, agt, att, cag, cat, ccg, cgg, cgt, cta, gaa, gct, ggt, gta, tgc, tgg, or ttt
  misc_feature (53)..(55): nnn = aac, act, agg, agt, att, cag, cat, ccg, cgg, cgt, cta, gaa, gct, ggt, gta, tgc, tgg, or ttt
  misc_feature (56)..(58): nnn = aac, act, agg, agt, att, cag, cat, ccg, cgg, cgt, cta, gaa, gct, ggt, gta, tgc, tgg, or ttt
  misc_feature (59)..(61): nnn = aac, act, agg, agt, att, cag, cat, ccg, cgg, cgt, cta, gaa, gct, ggt, gta, tgc, tgg, or ttt
  misc_feature (62)..(64): nnn = aac, act, agg, agt, att, cag, cat, ccg, cgg, cgt, cta, gaa, gct, ggt, gta, tgc, tgg, or ttt
  misc_feature (65)..(67): nnn = aac, act, agg, agt, att, cag, cat, ccg, cgg, cgt, cta, gaa, gct, ggt, gta, tgc, tgg, or ttt
  misc_feature (68)..(70): nnn = aac, act, agg, agt, att, cag, cat, ccg, cgg, cgt, cta, gaa, gct, ggt, gta, tgc, tgg, or ttt
  misc_feature (71)..(73): nnn = aac, act, agg, agt, att, cag, cat, ccg, cgg, cgt, cta, gaa, gct, ggt, gta, tgc, tgg, or ttt
  misc_feature (74)..(76): nnn = aac, act, agg, agt, att, cag, cat, ccg, cgg, cgt, cta, gaa, gct, ggt, gta, tgc, tgg, or ttt
gtaatacgactcactatagggttaactttaagaaggagatatacatatgnnnnnnnnnnnnnnnnnnnnnnnnnnnatgccgaccggcaccggcaccggcgatagggcggcggggacaaa

SEQ ID NO: 121 - DNA, 120 bp, Artificial Sequence
  v7c1 ID45_9 (TAG)
  misc_feature (50)..(52): nnn = aac, act, agg, agt, att, cag, cat, ccg, cgg, cgt, cta, gaa, gct, ggt, gta, tgc, tgg, or ttt
  misc_feature (53)..(55): nnn = aac, act, agg, agt, att, cag, cat, ccg, cgg, cgt, cta, gaa, gct, ggt, gta, tgc, tgg, or ttt
  misc_feature (56)..(58): nnn = aac, act, agg, agt, att, cag, cat, ccg, cgg, cgt, cta, gaa, gct, ggt, gta, tgc, tgg, or ttt
  misc_feature (59)..(61): nnn = aac, act, agg, agt, att, cag, cat, ccg, cgg, cgt, cta, gaa, gct, ggt, gta, tgc, tgg, or ttt
  misc_feature (62)..(64): nnn = aac, act, agg, agt, att, cag, cat, ccg, cgg, cgt, cta, gaa, gct, ggt, gta, tgc, tgg, or ttt
  misc_feature (65)..(67): nnn = aac, act, agg, agt, att, cag, cat, ccg, cgg, cgt, cta, gaa, gct, ggt, gta, tgc, tgg, or ttt
  misc_feature (68)..(70): nnn = aac, act, agg, agt, att, cag, cat, ccg, cgg, cgt, cta, gaa, gct, ggt, gta, tgc, tgg, or ttt
  misc_feature (71)..(73): nnn = aac, act, agg, agt, att, cag, cat, ccg, cgg, cgt, cta, gaa, gct, ggt, gta, tgc, tgg, or ttt
  misc_feature (74)..(76): nnn = aac, act, agg, agt, att, cag, cat, ccg, cgg, cgt, cta, gaa, gct, ggt, gta, tgc, tgg, or ttt
gtaatacgactcactatagggttaactttaagaaggagatatacatatgnnnnnnnnnnnnnnnnnnnnnnnnnnntagccgaccggcaccggcaccggcgatagggcggcggggacaaa

SEQ ID NO: 122 - RNA, 102 nt, Artificial Sequence
  v7c1 ID45_9 (ATG)
  misc_feature (32)..(34): nnn = aac, acu, agg, agu, auu, cag, cau, ccg, cgg, cgu, cua, gaa, gcu, ggu, gua, ugc, ugg, or uuu
  misc_feature (35)..(37): nnn = aac, acu, agg, agu, auu, cag, cau, ccg, cgg, cgu, cua, gaa, gcu, ggu, gua, ugc, ugg, or uuu
  misc_feature (38)..(40): nnn = aac, acu, agg, agu, auu, cag, cau, ccg, cgg, cgu, cua, gaa, gcu, ggu, gua, ugc, ugg, or uuu
  misc_feature (41)..(43): nnn = aac, acu, agg, agu, auu, cag, cau, ccg, cgg, cgu, cua, gaa, gcu, ggu, gua, ugc, ugg, or uuu
  misc_feature (44)..(46): nnn = aac, acu, agg, agu, auu, cag, cau, ccg, cgg, cgu, cua, gaa, gcu, ggu, gua, ugc, ugg, or uuu
  misc_feature (47)..(49): nnn = aac, acu, agg, agu, auu, cag, cau, ccg, cgg, cgu, cua, gaa, gcu, ggu, gua, ugc, ugg, or uuu
  misc_feature (50)..(52): nnn = aac, acu, agg, agu, auu, cag, cau, ccg, cgg, cgu, cua, gaa, gcu, ggu, gua, ugc, ugg, or uuu
  misc_feature (53)..(55): nnn = aac, acu, agg, agu, auu, cag, cau, ccg, cgg, cgu, cua, gaa, gcu, ggu, gua, ugc, ugg, or uuu
  misc_feature (56)..(58): nnn = aac, acu, agg, agu, auu, cag, cau, ccg, cgg, cgu, cua, gaa, gcu, ggu, gua, ugc, ugg, or uuu
ggguuaacuuuaagaaggagauauacauaugnnnnnnnnnnnnnnnnnnnnnnnnnnnaugccgaccggcaccggcaccggcgauagggcggcggggacaaa

SEQ ID NO: 123 - RNA, 102 nt, Artificial Sequence
  v7c1 ID45_9 (TAG)
  misc_feature (32)..(34): nnn = aac, acu, agg, agu, auu, cag, cau, ccg, cgg, cgu, cua, gaa, gcu, ggu, gua, ugc, ugg, or uuu
  misc_feature (35)..(37): nnn = aac, acu, agg, agu, auu, cag, cau, ccg, cgg, cgu, cua, gaa, gcu, ggu, gua, ugc, ugg, or uuu
  misc_feature (38)..(40): nnn = aac, acu, agg, agu, auu, cag, cau, ccg, cgg, cgu, cua, gaa, gcu, ggu, gua, ugc, ugg, or uuu
  misc_feature (41)..(43): nnn = aac, acu, agg, agu, auu, cag, cau, ccg, cgg, cgu, cua, gaa, gcu, ggu, gua, ugc, ugg, or uuu
  misc_feature (44)..(46): nnn = aac, acu, agg, agu, auu, cag, cau, ccg, cgg, cgu, cua, gaa, gcu, ggu, gua, ugc, ugg, or uuu
  misc_feature (47)..(49): nnn = aac, acu, agg, agu, auu, cag, cau, ccg, cgg, cgu, cua, gaa, gcu, ggu, gua, ugc, ugg, or uuu
  misc_feature (50)..(52): nnn = aac, acu, agg, agu, auu, cag, cau, ccg, cgg, cgu, cua, gaa, gcu, ggu, gua, ugc, ugg, or uuu
  misc_feature (53)..(55): nnn = aac, acu, agg, agu, auu, cag, cau, ccg, cgg, cgu, cua, gaa, gcu, ggu, gua, ugc, ugg, or uuu
  misc_feature (56)..(58): nnn = aac, acu, agg, agu, auu, cag, cau, ccg, cgg, cgu, cua, gaa, gcu, ggu, gua, ugc, ugg, or uuu
ggguuaacuuuaagaaggagauauacauaugnnnnnnnnnnnnnnnnnnnnnnnnnnnuagccgaccggcaccggcaccggcgauagggcggcggggacaaa

SEQ ID NO: 124 - protein, 12 aa, Artificial Sequence
  GS linker
GGGGSGGGSGGS